European Patent Application EP 4 382 133 A1, published June 12, 2024. Title: A pharmaceutical composition for treating triple negative breast cancer comprising a synthetic nucleic acid ligand as an active ingredient. Applicant: INTEROLIGO CORPORATION. Application WO. The sequence listing filed with the application follows.

SEQUENCE LISTING (17 sequences)

SEQ ID NO: 1 - DNA, 73 bp, synthetic construct
  source 1..73: mol_type = other DNA
  modified_base 21: mod_base = OTHER; note = 5-(N-(1-naphthylmethyl)carboxamide)-2-deoxyuridine
  modified_base 26: mod_base = OTHER; note = 5-(N-(1-naphthylmethyl)carboxamide)-2'-deoxyuridine
  modified_base 30: mod_base = OTHER; note = 5-(N-(1-naphthylmethyl)carboxamide)-2'-deoxyuridine
  modified_base 36: mod_base = OTHER; note = 5-(N-(1-naphthylmethyl)carboxamide)-2'-deoxyuridine
  modified_base 43..45: mod_base = OTHER; note = 5-(N-(1-naphthylmethyl)carboxamide)-2-deoxyuridine
  modified_base 47: mod_base = OTHER; note = 5-(N-(1-naphthylmethyl)carboxamide)-2'-deoxyuridine
  modified_base 56: mod_base = OTHER; note = 5-(N-(1-naphthylmethyl)carboxamide)-2'-deoxyuridine
gagtgaccgtctgcctggacnagcanaagnccgganggcagcnnnangccgaccancagccacaccaccagcc

SEQ ID NO: 2 - DNA, 49 bp, synthetic construct
  source 1..49: mol_type = other DNA
  modified_base 9: mod_base = OTHER; note = 5-(N-(1-naphthylmethyl)carboxamide)-2-deoxyuridine
  modified_base 14: mod_base = OTHER; note = 5-(N-(1-naphthylmethyl)carboxamide)-2'-deoxyuridine
  modified_base 18: mod_base = OTHER; note = 5-(N-(1-naphthylmethyl)carboxamide)-2'-deoxyuridine
  modified_base 24: mod_base = OTHER; note = 5-(N-(1-naphthylmethyl)carboxamide)-2'-deoxyuridine
  modified_base 31..33: mod_base = OTHER; note = 5-(N-(1-naphthylmethyl)carboxamide)-2'-deoxyuridine
  modified_base 35: mod_base = OTHER; note = 5-(N-(1-naphthylmethyl)carboxamide)-2'-deoxyuridine
  modified_base 44: mod_base = OTHER; note = 5-(N-(1-naphthylmethyl)carboxamide)-2'-deoxyuridine
gcctggacnagcanaagnccgganggcagcnnnangccgaccancagcc

SEQ ID NO: 3 - DNA, 39 bp, synthetic construct
  source 1..39: mol_type = other DNA
  modified_base 4: mod_base = OTHER; note = 5-(N-(1-naphthylmethyl)carboxamide)-2-deoxyuridine
  modified_base 9: mod_base = OTHER; note = 5-(N-(1-naphthylmethyl)carboxamide)-2'-deoxyuridine(Nap-dU)
  modified_base 13: mod_base = OTHER; note = 5-(N-(1-naphthylmethyl)carboxamide)-2'-deoxyuridine(Nap-dU)
  modified_base 19: mod_base = OTHER; note = 5-(N-(1-naphthylmethyl)carboxamide)-2'-deoxyuridine(Nap-dU)
  modified_base 26..28: mod_base = OTHER; note = 5-(N-(1-naphthylmethyl)carboxamide)-2'-deoxyuridine(Nap-dU)
  modified_base 30: mod_base = OTHER; note = 5-(N-(1-naphthylmethyl)carboxamide)-2'-deoxyuridine(Nap-dU)
  modified_base 39: mod_base = OTHER; note = 5-(N-(1-naphthylmethyl)carboxamide)-2'-deoxyuridine(Nap-dU)
gacnagcanaagnccgganggcagcnnnangccgaccan

SEQ ID NO: 4 - DNA, 34 bp, synthetic construct
  source 1..34: mol_type = other DNA
  modified_base 4: mod_base = OTHER; note = 5-(N-(1-naphthylmethyl)carboxamide)-2-deoxyuridine
  modified_base 9: mod_base = OTHER; note = 5-(N-(1-naphthylmethyl)carboxamide)-2'-deoxyuridine(Nap-dU)
  modified_base 13: mod_base = OTHER; note = 5-(N-(1-naphthylmethyl)carboxamide)-2'-deoxyuridine(Nap-dU)
  modified_base 19: mod_base = OTHER; note = 5-(N-(1-naphthylmethyl)carboxamide)-2'-deoxyuridine(Nap-dU)
  modified_base 26..28: mod_base = OTHER; note = 5-(N-(1-naphthylmethyl)carboxamide)-2'-deoxyuridine(Nap-dU)
  modified_base 30: mod_base = OTHER; note = 5-(N-(1-naphthylmethyl)carboxamide)-2'-deoxyuridine(Nap-dU)
gacnagcanaagnccgganggcagcnnnangccg

SEQ ID NO: 5 - DNA, 32 bp, synthetic construct
  source 1..32: mol_type = other DNA
  modified_base 4: mod_base = OTHER; note = 5-(N-(1-naphthylmethyl)carboxamide)-2-deoxyuridine(Nap-dU)
  modified_base 8: mod_base = OTHER; note = 5-(N-(1-naphthylmethyl)carboxamide)-2'-deoxyuridine(Nap-dU)
  modified_base 14: mod_base = OTHER; note = 5-(N-(1-naphthylmethyl)carboxamide)-2'-deoxyuridine(Nap-dU)
  modified_base 21..23: mod_base = OTHER; note = 5-(N-(1-naphthylmethyl)carboxamide)-2'-deoxyuridine(Nap-dU)
  modified_base 25: mod_base = OTHER; note = 5-(N-(1-naphthylmethyl)carboxamide)-2'-deoxyuridine(Nap-dU)
gcanaagnccgganggcagcnnnangccgacc

SEQ ID NO: 6 - DNA, 27 bp, synthetic construct
  source 1..27: mol_type = other DNA
  modified_base 4: mod_base = OTHER; note = 5-(N-(1-naphthylmethyl)carboxamide)-2'-deoxyuridine(Nap-dU)
  modified_base 8: mod_base = OTHER; note = 5-(N-(1-naphthylmethyl)carboxamide)-2'-deoxyuridine(Nap-dU)
  modified_base 14: mod_base = OTHER; note = 5-(N-(1-naphthylmethyl)carboxamide)-2'-deoxyuridine(Nap-dU)
  modified_base 21..23: mod_base = OTHER; note = 5-(N-(1-naphthylmethyl)carboxamide)-2'-deoxyuridine(Nap-dU)
  modified_base 25: mod_base = OTHER; note = 5-(N-(1-naphthylmethyl)carboxamide)-2'-deoxyuridine(Nap-dU)
gcanaagnccgganggcagcnnnangc

SEQ ID NO: 7 - DNA, 33 bp, synthetic construct
  source 1..33: mol_type = other DNA
  modified_base 4: mod_base = OTHER; note = 5-(N-(1-naphthylmethyl)carboxamide)-2'-deoxyuridine(Nap-dU)
  modified_base 9: mod_base = OTHER; note = 5-(N-(1-naphthylmethyl)carboxamide)-2'-deoxyuridine(Nap-dU)
  modified_base 13: mod_base = OTHER; note = 5-(N-(1-naphthylmethyl)carboxamide)-2'-deoxyuridine(Nap-dU
  modified_base 19: mod_base = OTHER; note = 5-(N-(1-naphthylmethyl)carboxamide)-2'-deoxyuridine(Nap-dU)
  modified_base 26..28: mod_base = OTHER; note = 5-(N-(1-naphthylmethyl)carboxamide)-2'-deoxyuridine(Nap-dU); note (original language) = 5-[N-(1-나프틸메틸)카복사마이드]-2'-데옥시우리딘(Nap-dU)
  modified_base 30: mod_base = OTHER; note = 5-(N-(1-naphthylmethyl)carboxamide)-2'-deoxyuridine(Nap-dU)
gacnagcanaagnccgganggcagcnnnangcc

SEQ ID NO: 8 - DNA, 43 bp, synthetic construct
  source 1..43: mol_type = other DNA
  modified_base 1..2: mod_base = OTHER; note = gemcitabine
  modified_base 8: mod_base = OTHER; note = 5-(N-(1-naphthylmethyl)carboxamide)-2'-deoxyuridine(Nap-dU)
  modified_base 13: mod_base = OTHER; note = 5-(N-(1-naphthylmethyl)carboxamide)-2'-deoxyuridine(Nap-dU)
  modified_base 17: mod_base = OTHER; note = 5-(N-(1-naphthylmethyl)carboxamide)-2'-deoxyuridine(Nap-dU)
  modified_base 23: mod_base = OTHER; note = 5-(N-(1-naphthylmethyl)carboxamide)-2'-deoxyuridine(Nap-dU)
  modified_base 30..32: mod_base = OTHER; note = 5-(N-(1-naphthylmethyl)carboxamide)-2'-deoxyuridine(Nap-dU)
  modified_base 34: mod_base = OTHER; note = 5-(N-(1-naphthylmethyl)carboxamide)-2'-deoxyuridine(Nap-dU)
  modified_base 43: mod_base = OTHER; note = 5-(N-(1-naphthylmethyl)carboxamide)-2'-deoxyuridine(Nap-dU)
nntggacnagcanaagnccgganggcagcnnnangccgaccan

SEQ ID NO: 9 - DNA, 39 bp, synthetic construct
  source 1..39: mol_type = other DNA
  modified_base 36..37: mod_base = OTHER; note = gemcitabine
  modified_base 39: mod_base = OTHER; note = 5-(N-(1-naphthylmethyl)carboxamide)-2'-deoxyuridine(Nap-dU)
  modified_base 30: mod_base = OTHER; note = 5-(N-(1-naphthylmethyl)carboxamide)-2'-deoxyuridine(Nap-dU)
  modified_base 26..28: mod_base = OTHER; note = 5-(N-(1-naphthylmethyl)carboxamide)-2'-deoxyuridine(Nap-dU)
  modified_base 19: mod_base = OTHER; note = 5-(N-(1-naphthylmethyl)carboxamide)-2'-deoxyuridine(Nap-dU)
  modified_base 13: mod_base = OTHER; note = 5-(N-(1-naphthylmethyl)carboxamide)-2'-deoxyuridine(Nap-dU)
  modified_base 9: mod_base = OTHER; note = 5-(N-(1-naphthylmethyl)carboxamide)-2'-deoxyuridine(Nap-dU)
  modified_base 4: mod_base = OTHER; note = 5-(N-(1-naphthylmethyl)carboxamide)-2'-deoxyuridine(Nap-dU)
gacnagcanaagnccgganggcagcnnnangccgannan

SEQ ID NO: 10 - DNA, 39 bp, synthetic construct
  source 1..39: mol_type = other DNA
  modified_base 3: mod_base = OTHER; note = Gemcitabine
  modified_base 7: mod_base = OTHER; note = gemcitabine
  modified_base 4: mod_base = OTHER; note = 5-(N-(1-naphthylmethyl)carboxamide)-2'-deoxyuridine(Nap-dU)
  modified_base 9: mod_base = OTHER; note = 5-(N-(1-naphthylmethyl)carboxamide)-2'-deoxyuridine(Nap-dU)
  modified_base 13: mod_base = OTHER; note = 5-(N-(1-naphthylmethyl)carboxamide)-2'-deoxyuridine(Nap-dU)
  modified_base 19: mod_base = OTHER; note = 5-(N-(1-naphthylmethyl)carboxamide)-2'-deoxyuridine(Nap-dU)
  modified_base 26..28: mod_base = OTHER; note = 5-(N-(1-naphthylmethyl)carboxamide)-2'-deoxyuridine(Nap-dU)
  modified_base 30: mod_base = OTHER; note = 5-(N-(1-naphthylmethyl)carboxamide)-2'-deoxyuridine(Nap-dU)
  modified_base 39: mod_base = OTHER; note = 5-(N-(1-naphthylmethyl)carboxamide)-2'-deoxyuridine(Nap-dU)
gannagnanaagnccgganggcagcnnnangccgaccan

SEQ ID NO: 11 - DNA, 27 bp, synthetic construct
  source 1..27: mol_type = other DNA
  modified_base 2: mod_base = OTHER; note = 2nd residue can be cystidine or gemcitabine
  modified_base 4: mod_base = OTHER; note = 5-(N-(1-naphthylmethyl)carboxamide)-2'-deoxyuridine(Nap-dU)
  modified_base 8: mod_base = OTHER; note = 5-(N-(1-naphthylmethyl)carboxamide)-2'-deoxyuridine(Nap-dU)
  modified_base 14: mod_base = OTHER; note = 5-(N-(1-naphthylmethyl)carboxamide)-2'-deoxyuridine(Nap-dU)
  modified_base 21..23: mod_base = OTHER; note = 5-(N-(1-naphthylmethyl)carboxamide)-2'-deoxyuridine(Nap-dU)
  modified_base 25: mod_base = OTHER; note = 5-(N-(1-naphthylmethyl)carboxamide)-2'-deoxyuridine(Nap-dU)
gnanaagnccgganggcagcnnnangc

SEQ ID NO: 12 - DNA, 74 bp, synthetic construct
  source 1..74: mol_type = other DNA
  misc_binding 1: bound_moiety = Biotin is biding to the 1st residue (5' end)
  misc_difference 17..56: note = The "n" can be replaced with the sequence of each nucleic acid ligand of the nucleic acid ligand library.
gctggtggtgtggctgnnnnnnnnnnnnnnnnnnnnnnnnnnnnnnnnnnnnnnnncaggcagacggtcactca

SEQ ID NO: 13 - DNA, 17 bp, synthetic construct
  source 1..17: mol_type = other DNA
gagtgaccgtctgcctg

SEQ ID NO: 14 - DNA, 16 bp, synthetic construct
  source 1..16: mol_type = other DNA
  misc_binding 1: bound_moiety = Biotin is binding to the 1st residue of the primer (5' end)
gctggtggtgtggctg

SEQ ID NO: 15 - DNA, 17 bp, synthetic construct
  source 1..17: mol_type = other DNA
  misc_binding 1: bound_moiety = Biotin is biding to the 1st residue of the primer (5' end)
gagtgaccgtctgcctg

SEQ ID NO: 16 - DNA, 16 bp, synthetic construct
  source 1..16: mol_type = other DNA
gctggtggtgtggctg

SEQ ID NO: 17 - DNA, 40 bp, synthetic construct
  source 1..40: mol_type = other DNA
  modified_base 2: mod_base = OTHER; note = 5-(N-(1-naphthylmethyl)carboxamide)-2'-deoxyuridine(Nap-dU)
  modified_base 4..5: mod_base = OTHER; note = 5-(N-(1-naphthylmethyl)carboxamide)-2'-deoxyuridine(Nap-dU)
  modified_base 10..12: mod_base = OTHER; note = 5-(N-(1-naphthylmethyl)carboxamide)-2'-deoxyuridine(Nap-dU)
  modified_base 16: mod_base = OTHER; note = 5-(N-(1-naphthylmethyl)carboxamide)-2'-deoxyuridine(Nap-dU)
  modified_base 20: mod_base = OTHER; note = 5-(N-(1-naphthylmethyl)carboxamide)-2'-deoxyuridine(Nap-dU)
  modified_base 24: mod_base = OTHER; note = 5-(N-(1-naphthylmethyl)carboxamide)-2'-deoxyuridine(Nap-dU)
  modified_base 35: mod_base = OTHER; note = 5-(N-(1-naphthylmethyl)carboxamide)-2'-deoxyuridine(Nap-dU)
angnnagagnnngccngagngccncgcaagggcgnaacaa